European Patent Specification EP 3 908 604 B1, published July 3, 2024. Title: GALECTIN-7-SPECIFIC MONOVALENT ANTIBODIES AND USES THEREOF. Applicant: INSTITUT NATIONAL DE LA RECHERCHE SCIENTIFIQUE. The sequence listing filed with the application follows.

SEQUENCE LISTING (54 sequences)

SEQ ID NO: 1 - protein, 121 aa, Artificial Sequence
  Humanized synthetic single domain antibody
MAEVQLQASGGGFVQPGGSLRLSCAASGAGSRSDVMGWFRQAPGKEREFVSAISGFWGWTTYYADSVKGRFTISRDNSKNTVYLQMNSLRAEDTATYYCALGGAPGQTGYWGQGTQVTVSS

SEQ ID NO: 2 - protein, 124 aa, Artificial Sequence
  Humanized synthetic single domain antibody
MAEVQLQASGGGFVQPGGSLRLSCAASGDTSRFDVMGWFRQAPGKEREFVSAISWWSSDHIYYADSVKGRFTISRDNSKNTVYLQMNSLRAEDTATYYCAYGEYPPRMNRRPYWGQGTQVTVSS

SEQ ID NO: 3 - protein, 127 aa, Artificial Sequence
  Humanized synthetic single domain antibody
MAEVQLQASGGGFVQPGGSLRLSCAASGTTSNSSGMGWFRQAPGKEREFVSAISWDHGILTYYADSVKGRFTISRDNSKNTVYLQMNSLRAEDTATYYCAHGYVHFNMTHRHISDYWGQGTQVTVSS

SEQ ID NO: 4 - protein, 124 aa, Artificial Sequence
  Humanized synthetic single domain antibody
MAEVQLQASGGGFVQPGGSLRLSCAASGTTSNGEVMGWFRQAPGKEREFVSAISFGAGSSEYYADSVKGRFTISRDNSKNTVYLQMNSLRAEDTATYYCAASWYHSSIGSMSYWGQGTQVTVSS

SEQ ID NO: 5 - protein, 121 aa, Artificial Sequence
  Humanized synthetic single domain antibody
MAEVQLQASGGGFVQPGGSLRLSCAASGAYSFESGMGWFRQAPGKEREFVSAISSDADLFSYYADSVKGRFTISRDNSKNTVYLQMNSLRAEDTATYYCAAFSSGGELSYWGQGTQVTVSS

SEQ ID NO: 6 - protein, 121 aa, Artificial Sequence
  Humanized synthetic single domain antibody
MAEVQLQASGGGFVQPGGSLRLSCAASGRYSRIEIMGWFRQAPGKEREFVSAISSTPSSNEYYADSVKGRFTISRDNSKNTVYLQMNSLRAEDTATYYCARWDWHSWDTYWGQGTQVTVSS

SEQ ID NO: 7 - protein, 130 aa, Artificial Sequence
  Humanized synthetic single domain antibody
MAEVQLQASGGGFVQPGGSLRLSCAASGSTSYSSTMGWFRQAPGKEREFVSAISFDGTSKPYYADSVKGRFTISRDNSKNTVYLQMNSLRAEDTATYYCAAGEWEALMWPPVHDFWIYYWGQGTQVTVSS

SEQ ID NO: 8 - protein, 121 aa, Artificial Sequence
  Humanized synthetic single domain antibody
MAEVQLQASGGGFVQPGGSLRLSCAASGRTSSQDIMGWFRQAPGKEREFVSAISDYSGGNVYYADSVKGRFTISRDNSKNTVYLQMNSLRAEDTATYYCAFLGEEKTSWYWGQGTQVTVSS

SEQ ID NO: 9 - protein, 130 aa, Artificial Sequence
  Humanized synthetic single domain antibody
MAEVQLQASGGGFVQPGGSLRLSCAASGSTSYGETMGWFRQAPGKEREFVSAISYYSTRKPYYADSVKGRFTISRDNSKNTVYLQMNSLRAEDTATYYCAIVAYIYADGVRGYHQKIDYWGQGTQVTVSS

SEQ ID NO: 10 - protein, 115 aa, Artificial Sequence
  Humanized synthetic single domain antibody
MAEVQLQASGGGFVQPGGSLRLSCAASGGGYDWDAMGWFRQAPGKEREFVSAISSNNNGSRYYADSVKGRFTISRDNSKNTVYLQMNSLRAEDTATYYCAADQYWGQGTQVTVSS

SEQ ID NO: 11 - protein, 121 aa, Artificial Sequence
  Humanized synthetic single domain antibody
  VARIANT (29)..(35): Xaa at each of residues 29 to 35 is any amino acid
  VARIANT (55)..(61): Xaa at each of residues 55 to 61 is any amino acid
  VARIANT (101)..(109): Xaa at each of residues 101 to 109 is any amino acid
MAEVQLQASGGGFVQPGGSLRLSCAASGXXXXXXXMGWFRQAPGKEREFVSAISXXXXXXXYYADSVKGRFTISRDNSKNTVYLQMNSLRAEDTATYYCAXXXXXXXXXYWGQGTQVTVSS

SEQ ID NO: 12 - protein, 7 aa, Artificial Sequence
  CDR1 domain
AGSRSDV

SEQ ID NO: 13 - protein, 7 aa, Artificial Sequence
  CDR2 domain
GFWGWTT

SEQ ID NO: 14 - protein, 9 aa, Artificial Sequence
  CDR3 domain
LGGAPGQTG

SEQ ID NO: 15 - protein, 7 aa, Artificial Sequence
  CDR1 domain
DTSRFDV

SEQ ID NO: 16 - protein, 7 aa, Artificial Sequence
  CDR2 domain
WWSSDHI

SEQ ID NO: 17 - protein, 12 aa, Artificial Sequence
  CDR3 domain
YGEYPPRMNRRP

SEQ ID NO: 18 - protein, 7 aa, Artificial Sequence
  CDR1 domain
TTSNSSG

SEQ ID NO: 19 - protein, 7 aa, Artificial Sequence
  CDR2 domain
WDHGILT

SEQ ID NO: 20 - protein, 15 aa, Artificial Sequence
  CDR3 domain
HGYVHFNMTHRHISD

SEQ ID NO: 21 - protein, 7 aa, Artificial Sequence
  CDR1 domain
TTSNGEV

SEQ ID NO: 22 - protein, 7 aa, Artificial Sequence
  CDR2 domain
FGAGSSE

SEQ ID NO: 23 - protein, 12 aa, Artificial Sequence
  CDR3 domain
ASWYHSSIGSMS

SEQ ID NO: 24 - protein, 7 aa, Artificial Sequence
  CDR1 domain
AYSFESG

SEQ ID NO: 25 - protein, 7 aa, Artificial Sequence
  CDR2 domain
SDADLFS

SEQ ID NO: 26 - protein, 9 aa, Artificial Sequence
  CDR3 domain
AFSSGGELS

SEQ ID NO: 27 - protein, 7 aa, Artificial Sequence
  CDR1 domain
RYSRIEI

SEQ ID NO: 28 - protein, 7 aa, Artificial Sequence
  CDR2 domain
STPSSNE

SEQ ID NO: 29 - protein, 9 aa, Artificial Sequence
  CDR3 domain
RWDWHSWDT

SEQ ID NO: 30 - protein, 7 aa, Artificial Sequence
  CDR1 domain
STSYSST

SEQ ID NO: 31 - protein, 7 aa, Artificial Sequence
  CDR2 domain
FDGTSKP

SEQ ID NO: 32 - protein, 18 aa, Artificial Sequence
  CDR3 domain
AGEWEALMWPPVHDFWIY

SEQ ID NO: 33 - protein, 7 aa, Artificial Sequence
  CDR1 domain
RTSSQDI

SEQ ID NO: 34 - protein, 7 aa, Artificial Sequence
  CDR2 domain
DYSGGNV

SEQ ID NO: 35 - protein, 9 aa, Artificial Sequence
  CDR3 DOMAIN
FLGEEKTSW

SEQ ID NO: 36 - protein, 7 aa, Artificial Sequence
  CDR1 domain
STSYGET

SEQ ID NO: 37 - protein, 7 aa, Artificial Sequence
  CDR2 domain
YYSTRKP

SEQ ID NO: 38 - protein, 18 aa, Artificial Sequence
  CDR3 domain
IVAYIYADGVRGYHQKID

SEQ ID NO: 39 - protein, 7 aa, Artificial Sequence
  CDR1 domain
GGYDWDA

SEQ ID NO: 40 - protein, 7 aa, Artificial Sequence
  CDR2 domain
SNNNGSR

SEQ ID NO: 41 - protein, 4 aa, Artificial Sequence
  CDR3 DOMAIN
  MISC (4)..(4): X at position 4 is absent
ADQX

SEQ ID NO: 42 - protein, 7 aa, Artificial Sequence
  CDR1 domain
TYSSIEV

SEQ ID NO: 43 - protein, 7 aa, Artificial Sequence
  CDR2 domain
FEPNEFA

SEQ ID NO: 44 - protein, 15 aa, Artificial Sequence
  CDR3 domain
SSVEWRQNGKPNTAS

SEQ ID NO: 45 - protein, 7 aa, Artificial Sequence
  CDR1 domain
DTSESTS

SEQ ID NO: 46 - protein, 7 aa, Artificial Sequence
  CDR2 domain
RSSTWDA

SEQ ID NO: 47 - protein, 15 aa, Artificial Sequence
  CDR3 domain
MADIFDHPQNASFMK

SEQ ID NO: 48 - protein, 28 aa, Artificial Sequence
  FR1 domain
MAEVQLQASGGGFVQPGGSLRLSCAASG

SEQ ID NO: 49 - protein, 19 aa, Artificial Sequence
  FR2 domain
MGWFRQAPGKEREFVSAIS

SEQ ID NO: 50 - protein, 39 aa, Artificial Sequence
  FR3 domain
YYADSVKGRFTISRDNSKNTVYLQMNSLRAEDTATYYCA

SEQ ID NO: 51 - protein, 12 aa, Artificial Sequence
  FR4 domain
YWGQGTQVTVSS

SEQ ID NO: 52 - protein, 127 aa, Artificial Sequence
  Recombinant antibody
MAEVQLQASGGGFVQPGGSLRLSCAASGTYSSIEVMGWFRQAPGKEREFVSAISFEPNEFAYYADSVKGRFTISRDNSKNTVYLQMNSLRAEDTATYYCASSVEWRQNGKPNTASYWGQGTQVTVSS

SEQ ID NO: 53 - protein, 127 aa, Artificial Sequence
  Recombinant antibody
MAEVQLQASGGGFVQPGGSLRLSCAASGDTSESTSMGWFRQAPGKEREFVSAISRSSTWDAYYADSVKGRFTISRDNSKNTVYLQMNSLRAEDTATYYCAMADIFDHPQNASFMKYWGQGTQVTVSS

SEQ ID NO: 54 - protein, 54 aa, Artificial Sequence
  Synthetic tag
AAAHHHHHHGAAEQKLISEEDLNGAAEQKLISEEDLNGAAEQKLISEEDLNGAA